European Patent Application EP 4 556 553 A1, published May 21, 2025. Title: A novel Schizochytrium sp. strain producing a biomass containing high protein content, antioxidant pigments and omega-3 fatty acid and use thereof. Applicant: CJ CheilJedang Corporation. Application KR. The sequence listing filed with the application follows.

SEQUENCE LISTING (5 sequences)

SEQ ID NO: 1 - DNA, 137 bp, synthetic construct
  source 1..137: mol_type = other DNA
tttcagactgctttttgctttttgcttgcttgctttttgcttgcttgcttttggcttgctttctttttgcttcttcctgcttgatccggtgaagaagaacggagcgaactaaaagaaaagagtcaatccgaagagag

SEQ ID NO: 2 - DNA, 122 bp, synthetic construct
  source 1..122: mol_type = other DNA
tttcagactgctttttgctttttgcttgcttgcttttggcttgctttctttttgcttcttcctgcttgatccggtgaagaagaacggagcgaactaaaagaaaagagtcaatccgaagagag

SEQ ID NO: 3 - DNA, 24 bp, synthetic construct
  source 1..24: mol_type = other DNA
tttcagactgctttttgctttttg

SEQ ID NO: 4 - DNA, 24 bp, synthetic construct
  source 1..24: mol_type = other DNA
ctctcttcggattgactcttttct

SEQ ID NO: 5 - DNA, 15 bp, synthetic construct
  source 1..15: mol_type = other DNA
tgcttgcttgctttt